European Patent Specification EP 3 791 859 B1, published August 26, 2026. Title: FORMULATIONS FOR SMALL INTESTINAL DELIVERY OF RSV AND NOROVIRUS ANTIGENS. Applicant: Vaxart, Inc. The sequence listing filed with the application follows.

SEQUENCE LISTING (11 sequences)

SEQ ID NO: 1 - DNA, 1593 bp, Artificial Sequence
  synthetic nucleotide sequence - Codon optimized DNA encoding the 58 kd capsid protein [Norwalk virus] (insert in VXA-G1.1-NN)
atgatgatggcgagtaaagacgctacatcctccgtggatggggcctctggagcaggtcagctggtgccggaggtgaacgcatcagatcctcttgctatggacccagtggcaggaagcagtactgcagtcgctactgctggacaagtaaatcccatcgatccctggatcatcaataacttcgtgcaggccccacaaggcgaatttactatttcccccaacaacacgcctggcgatgtgttgttcgatctgtctcttggcccccatctgaacccctttctgttgcatctctcccagatgtacaatggctgggtgggcaatatgcgcgtgcgcattatgttggccggtaacgcgtttacagctggaaaaataatcgtgagctgcattcctcccggcttcggttcccataatctgacaatagcgcaggctaccctgttccctcacgtgatcgcggatgtgagaacacttgatcccatagaggtgcctctggaagacgtgagaaatgtcttgttccataataatgaccggaatcaacaaacaatgaggctggtgtgcatgttgtacacacctctgcggacgggcggcggaacaggggactcatttgtagtggcaggaagagtgatgacctgcccttctcccgacttcaatttcctgtttttggttcctcccacagtcgagcagaagactaggccatttaccctgcccaatctcccgcttagctcactgtctaattcaagagcaccgctgccaatttcttcaatgggcatttccccggacaatgtgcagtccgttcaattccagaacggcaggtgtacgctggatggcagacttgtcggcactacaccggtcagcctctcacacgttgccaaaattcggggtacttccaacggcacggtcatcaacttgaccgagctggacgggaccccgttccacccctttgagggccccgctcctatcgggtttcccgatctgggagggtgtgattggcacatcaacatgacacagtttgggcatagctcacagacgcagtacgacgtcgataccacccctgacacattcgtgccgcatctcggctcaatccaggcaaacggcatagggagtggtaattatgtcggtgtcttgagttggatctctccgccctctcacccttccggttcccaagtagacctctggaagatccccaattacggctcctctatcaccgaggccacccacttggccccatccgtctatcccccaggattcggggaggtactcgttttcttcatgagtaagatgcctggtcctggcgcctacaatctgccttgcttgttgccccaggagtacattagccacctggcctctgaacaggcccccaccgtgggagaagccgctttgttgcattacgtcgaccccgacaccggtagaaacctgggagagtttaaagcatatcctgatgggttccttacctgcgtgcccaatggcgcatcatctggcccccagcagctgccgatcaatggcgttttcgtctttgtgtcctgggtatcccgcttctaccagctgaagccggttggcacagcctcatcagcacgcggcagactgggcctcagaagataa

SEQ ID NO: 2 - protein, 530 aa, Unknown
  Norwalk virus - 58 kd capsid protein
MMMASKDATSSVDGASGAGQLVPEVNASDPLAMDPVAGSSTAVATAGQVNPIDPWIINNFVQAPQGEFTISPNNTPGDVLFDLSLGPHLNPFLLHLSQMYNGWVGNMRVRIMLAGNAFTAGKIIVSCIPPGFGSHNLTIAQATLFPHVIADVRTLDPIEVPLEDVRNVLFHNNDRNQQTMRLVCMLYTPLRTGGGTGDSFVVAGRVMTCPSPDFNFLFLVPPTVEQKTRPFTLPNLPLSSLSNSRAPLPISSMGISPDNVQSVQFQNGRCTLDGRLVGTTPVSLSHVAKIRGTSNGTVINLTELDGTPFHPFEGPAPIGFPDLGGCDWHINMTQFGHSSQTQYDVDTTPDTFVPHLGSIQANGIGSGNYVGVLSWISPPSHPSGSQVDLWKIPNYGSSITEATHLAPSVYPPGFGEVLVFFMSKMPGPGAYNLPCLLPQEYISHLASEQAPTVGEAALLHYVDPDTGRNLGEFKAYPDGFLTCVPNGASSGPQQLPINGVFVFVSWVSRFYQLKPVGTASSARGRLGLRR

SEQ ID NO: 3 - DNA, 1623 bp, Artificial Sequence
  synthetic nucleotide sequence - Codon Optimized sequence encoding Norovirus Hu/GII.4/Sydney/NSW0514/2012/AU  (insert in VXA-G2.4-NS)
atgaagatggctagcagcgatgccaatccgagtgatgggtccgcagccaatctggtcccggaggttaacaatgaagtgatggctctggaacctgtggtgggtgctgcaatcgccgcacctgttgcagggcagcagaacgttattgatccctggatcaggaacaacttcgtgcaagcacccggcggtgaattcaccgtgagccccaggaacgccccaggcgaaattctgtggtctgccccactggggcctgatctgaacccctatctgtctcacctggcaagaatgtataacgggtatgccggagggtttgaggtccaggtcatcctggcgggaaacgcctttactgcaggcaaggtgatatttgcggccgtacctcccaattttccaaccgagggacttagcccatcccaggtgacaatgtttcctcacatcgtggtcgatgtgcgccagcttgagccagtcctgattccactgccagacgtgagaaataacttttatcattacaatcaatcaaacgacccaaccatcaaactgatcgccatgctgtacactcctcttcgcgccaacaacgctggtgacgatgtgtttacagtgtcttgtcgggtcctcactcgcccctccccagattttgactttatttttctcgtgccgccaacggttgaaagtaggacaaagcctttctccgtaccagtgctcactgtggaggagatgaccaacagccggtttccgatccctctggagaaactgttcacggggccttctagtgctttcgtggttcagccacaaaacgggaggtgcaccacagatggcgtactgcttgggactacccagcttagccccgtgaatatttgtaccttccggggggatgtgacacacattaccggctccaggaactataccatgaatctggcctcccaaaattggaacgactatgatcccaccgaggagatccctgcccctctgggcactcctgactttgttggaaagatacagggcgtcctgacacaaacaacaagaaccgatggctctacccgggggcataaggcaaccgtgtacactgggtccgctgactttgcgcccaaactgggacgggtccaattcgagactgacacagaccgagacttcgaggcgaatcagaacacaaagttcacccctgtcggtgtgattcaggacgggggcaccactcatcggaacgagccccaacagtgggtcttgccctcctactccgggaggaatactcacaatgttcacctggcccccgccgtggcccccacgttcccaggtgaacaactgctgttttttagatctactatgcctggttgttccggctatccaaacatggaccttgattgtctgctgccacaggagtgggtgcagtatttctaccaggaagcagccccagcccagtcagatgttgccttgcttcggttcgtgaatcctgataccgggagggttctcttcgaatgcaagctgcacaaatctggctacgtgacggtagcgcatactggacagcatgacctcgtcattcccccaaacggatactttcgattcgatagctgggtaaaccagttttatacactggcacctatgggcaacgggaccggcaggaggcgggcggtgtaa

SEQ ID NO: 4 - protein, 540 aa, Unknown
  Norovirus Hu/GII.4/Sydney/NSW0514/2012/AU
MKMASSDANPSDGSAANLVPEVNNEVMALEPVVGAAIAAPVAGQQNVIDPWIRNNFVQAPGGEFTVSPRNAPGEILWSAPLGPDLNPYLSHLARMYNGYAGGFEVQVILAGNAFTAGKVIFAAVPPNFPTEGLSPSQVTMFPHIVVDVRQLEPVLIPLPDVRNNFYHYNQSNDPTIKLIAMLYTPLRANNAGDDVFTVSCRVLTRPSPDFDFIFLVPPTVESRTKPFSVPVLTVEEMTNSRFPIPLEKLFTGPSSAFVVQPQNGRCTTDGVLLGTTQLSPVNICTFRGDVTHITGSRNYTMNLASQNWNDYDPTEEIPAPLGTPDFVGKIQGVLTQTTRTDGSTRGHKATVYTGSADFAPKLGRVQFETDTDRDFEANQNTKFTPVGVIQDGGTTHRNEPQQWVLPSYSGRNTHNVHLAPAVAPTFPGEQLLFFRSTMPGCSGYPNMDLDCLLPQEWVQYFYQEAAPAQSDVALLRFVNPDTGRVLFECKLHKSGYVTVAHTGQHDLVIPPNGYFRFDSWVNQFYTLAPMGNGTGRRRAV

SEQ ID NO: 5 - DNA, 1725 bp, Artificial Sequence
  synthetic nucleotide sequence - Codon optimized sequence for the RSV A2 Fusion glycoprotein F0
atggagctgcccatccttaaggcaaatgccattacgacaatcctggcggccgtcaccttctgctttgccagctcacagaatatcactgaggagttttaccagtctacatgttcagcggtctccaaagggtacttgagtgcgctccgaaccggatggtacacaagcgtcatcaccatagaactgtccaatataaaggagaataaatgcaatgggaccgatgcaaaagttaaactcatcaaacaggaactcgacaagtacaagaatgccgtgacggagctccagctgctgatgcagtctacacctgcagctaacaacagggcaaggcgcgaactcccaagattcatgaattatacactgaacaacacgaagaagaccaatgttacactgagcaagaaacgaaagcgccgctttctcggatttcttcttggcgtagggtccgccatcgcatcaggtatcgcagtgagcaaagttctccatctcgagggcgaggtaaacaagataaaatccgcattgctcagcaccaacaaggctgtggtgtccttgagcaatggcgtatcagtgctgaccagcaaggttctggatctcaagaactatattgacaaacagctgctgcctattgtgaacaagcagtcttgtagaattagcaacatcgagaccgtcattgagttccagcagaaaaataatagattgctggagatcacgcgggagttcagcgttaatgctggagtcacaacccctgttagcacgtatatgctgaccaacagcgagttgcttagcttgatcaatgatatgccgataacgaatgatcagaagaaattgatgtccaacaatgtccagatcgtgcgacagcagagctactccatcatgtcaattatcaaggaggaagtgctcgcatacgtggtccagctcccattgtacggcgtgatcgacactccatgctggaagctgcacacatcacctctgtgcaccactaacactaaagaaggttcaaatatctgtctcacaaggaccgaccgagggtggtattgcgataacgctggatctgtgagttttttccctcaggctgagacatgcaaagtgcaaagcaaccgagtattctgtgacacaatgaactcacttaccctcccatccgaggtgaatctctgtaacgtggacatatttaaccctaagtacgattgtaagatcatgacctctaaaacagatgtcagtagttctgtgattaccagtttgggtgcaatagtcagctgctatgggaaaactaaatgtacagcttctaataagaaccgagggatcatcaagaccttctctaatggatgtgactatgttagcaacaagggggttgacacagtgtccgtaggcaacactctgtattatgtaaacaagcaggaaggaaaaagtctctacgtcaagggagaaccgatcattaatttctacgatccgttggtcttcccctccgatgaattcgacgcgagtatatcccaggtcaatgagaaaattaatcagagccttgcttttatcaggaagagtgatgagcttctccaccatgtcaatgctggcaaatccacaacaaacatcatgatcactaccatcatcatcgtgatcattgtgattctcttgagcctcatcgctgttggactgcttctgtactgtaaggcacgctctactcctgttactctctccaaagatcagctctccggtatcaataatatcgcatttagcaattga

SEQ ID NO: 6 - protein, 566 aa, respiratory syncytial virus
  MISC_FEATURE (1)..(566): RSV A2 Fusion glycoprotein F0
MELPILKANAITTILAAVTFCFASSQNITEEFYQSTCSAVSKGYLSALRTGWYTSVITIELSNIKENKCNGTDAKVKLIKQELDKYKNAVTELQLLMQSTPAANNRARRELPRFMNYTLNNTKKTNVTLSKKRKRRFLGFLLGVGSAIASGIAVSKVLHLEGEVNKIKSALLSTNKAVVSLSNGVSVLTSKVLDLKNYIDKQLLPIVNKQSCRISNIETVIEFQQKNNRLLEITREFSVNAGVTTPVSTYMLTNSELLSLINDMPITNDQKKLMSNNVQIVRQQSYSIMSIIKEEVLAYVVQLPLYGVIDTPCWKLHTSPLCTTNTKEGSNICLTRTDRGWYCDNAGSVSFFPQAETCKVQSNRVFCDTMNSLTLPSEVNLCNVDIFNPKYDCKIMTSKTDVSSSVITSLGAIVSCYGKTKCTASNKNRGIIKTFSNGCDYVSNKGVDTVSVGNTLYYVNKQEGKSLYVKGEPIINFYDPLVFPSDEFDASISQVNEKINQSLAFIRKSDELLHHVNAGKSTTNIMITTIIIVIIVILLSLIAVGLLLYCKARSTPVTLSKDQLSG

SEQ ID NO: 7 - DNA, 30098 bp, Artificial Sequence
  synthetic nucleotide sequence - Adenoviral vector backbone
  misc_feature (30089)..(30093): n is a, c, g or t
taaggatcccatcatcaataatataccttattttggattgaagccaatatgataatgagggggtggagtttgtgacgtggcgcggggcgtgggaacggggcgggtgacgtagtagtgtggcggaagtgtgatgttgcaagtgtggcggaacacatgtaagcgacggatgtggcaaaagtgacgtttttggtgtgcgccggtgtacacaggaagtgacaattttcgcgcggttttaggcggatgttgtagtaaatttgggcgtaaccgagtaagatttggccattttcgcgggaaaactgaataagaggaagtgaaatctgaataattttgtgttactcatagcgcgtaatgtgggaaagaatatataaggtgggggtcttatgtagttttgtatctgttttgcagcagccgccgccgccatgagcaccaactcgtttgatggaagcattgtgagctcatatttgacaacgcgcatgcccccatgggccggggtgcgtcagaatgtgatgggctccagcattgatggtcgccccgtcctgcccgcaaactctactaccttgacctacgagaccgtgtctggaacgccgttggagactgcagcctccgccgccgcttcagccgctgcagccaccgcccgcgggattgtgactgactttgctttcctgagcccgcttgcaagcagtgcagcttcccgttcatccgcccgcgatgacaagttgacggctcttttggcacaattggattctttgacccgggaacttaatgtcgtttctcagcagctgttggatctgcgccagcaggtttctgccctgaaggcttcctcccctcccaatgcggtttaaaacataaataaaaaaccagactctgtttggatttggatcaagcaagtgtcttgctgtctttatttaggggttttgcgcgcgcggtaggcccgggaccagcggtctcggtcgttgagggtcctgtgtattttttccaggacgtggtaaaggtgactctggatgttcagatacatgggcataagcccgtctctggggtggaggtagcaccactgcagagcttcatgctgcggggtggtgttgtagatgatccagtcgtagcaggagcgctgggcgtggtgcctaaaaatgtctttcagtagcaagctgattgccaggggcaggcccttggtgtaagtgtttacaaagcggttaagctgggatgggtgcatacgtggggatatgagatgcatcttggactgtatttttaggttggctatgttcccagccatatccctccggggattcatgttgtgcagaaccaccagcacagtgtatccggtgcacttgggaaatttgtcatgtagcttagaaggaaatgcgtggaagaacttggagacgcccttgtgacctccaagattttccatgcattcgtccataatgatggcaatgggcccacgggcggcggcctgggcgaagatatttctgggatcactaacgtcatagttgtgttccaggatgagatcgtcataggccatttttacaaagcgcgggcggagggtgccagactgcggtataatggttccatccggcccaggggcgtagttaccctcacagatttgcatttcccacgctttgagttcagatggggggatcatgtctacctgcggggcgatgaagaaaacggtttccggggtaggggagatcagctgggaagaaagcaggttcctgagcagctgcgacttaccgcagccggtgggcccgtaaatcacacctattaccgggtgcaactggtagttaagagagctgcagctgccgtcatccctgagcaggggggccacttcgttaagcatgtccctgactcgcatgttttccctgaccaaatccgccagaaggcgctcgccgcccagcgatagcagttcttgcaaggaagcaaagtttttcaacggtttgagaccgtccgccgtaggcatgcttttgagcgtttgaccaagcagttccaggcggtcccacagctcggtcacctgctctacggcatctcgatccagcatatctcctcgtttcgcgggttggggcggctttcgctgtacggcagtagtcggtgctcgtccagacgggccagggtcatgtctttccacgggcgcagggtcctcgtcagcgtagtctgggtcacggtgaaggggtgcgctccgggctgcgcgctggccagggtgcgcttgaggctggtcctgctggtgctgaagcgctgccggtcttcgccctgcgcgtcggccaggtagcatttgaccatggtgtcatagtccagcccctccgcggcgtggcccttggcgcgcagcttgcccttggaggaggcgccgcacgaggggcagtgcagacttttgagggcgtagagcttgggcgcgagaaataccgattccggggagtaggcatccgcgccgcaggccccgcagacggtctcgcattccacgagccaggtgagctctggccgttcggggtcaaaaaccaggtttcccccatgctttttgatgcgtttcttacctctggtttccatgagccggtgtccacgctcggtgacgaaaaggctgtccgtgtccccgtatacagacttgagaggcctgtcctcgagcggtgttccgcggtcctcctcgtatagaaactcggaccactctgagacaaaggctcgcgtccaggccagcacgaaggaggctaagtgggaggggtagcggtcgttgtccactagggggtccactcgctccagggtgtgaagacacatgtcgccctcttcggcatcaaggaaggtgattggtttgtaggtgtaggccacgtgaccgggtgttcctgaaggggggctataaaagggggtgggggcgcgttcgtcctcactctcttccgcatcgctgtctgcgagggccagctgttggggtgagtactccctctgaaaagcgggcatgacttctgcgctaagattgtcagtttccaaaaacgaggaggatttgatattcacctggcccgcggtgatgcctttgagggtggccgcatccatctggtcagaaaagacaatctttttgttgtcaagcttggtggcaaacgacccgtagagggcgttggacagcaacttggcgatggagcgcagggtttggtttttgtcgcgatcggcgcgctccttggccgcgatgtttagctgcacgtattcgcgcgcaacgcaccgccattcgggaaagacggtggtgcgctcgtcgggcaccaggtgcacgcgccaaccgcggttgtgcagggtgacaaggtcaacgctggtggctacctctccgcgtaggcgctcgttggtccagcagaggcggccgcccttgcgcgagcagaatggcggtagggggtctagctgcgtctcgtccggggggtctgcgtccacggtaaagaccccgggcagcaggcgcgcgtcgaagtagtctatcttgcatccttgcaagtctagcgcctgctgccatgcgcgggcggcaagcgcgcgctcgtatgggttgagtgggggaccccatggcatggggtgggtgagcgcggaggcgtacatgccgcaaatgtcgtaaacgtagaggggctctctgagtattccaagatatgtagggtagcatcttccaccgcggatgctggcgcgcacgtaatcgtatagttcgtgcgagggagcgaggaggtcgggaccgaggttgctacgggcgggctgctctgctcggaagactatctgcctgaagatggcatgtgagttggatgatatggttggacgctggaagacgttgaagctggcgtctgtgagacctaccgcgtcacgcacgaaggaggcgtaggagtcgcgcagcttgttgaccagctcggcggtgacctgcacgtctagggcgcagtagtccagggtttccttgatgatgtcatacttatcctgtcccttttttttccacagctcgcggttgaggacaaactcttcgcggtctttccagtactcttggatcggaaacccgtcggcctccgaacggtaagagcctagcatgtagaactggttgacggcctggtaggcgcagcatcccttttctacgggtagcgcgtatgcctgcgcggccttccggagcgaggtgtgggtgagcgcaaaggtgtccctgaccatgactttgaggtactggtatttgaagtcagtgtcgtcgcatccgccctgctcccagagcaaaaagtccgtgcgctttttggaacgcggatttggcagggcgaaggtgacatcgttgaagagtatctttcccgcgcgaggcataaagttgcgtgtgatgcggaagggtcccggcacctcggaacggttgttaattacctgggcggcgagcacgatctcgtcaaagccgttgatgttgtggcccacaatgtaaagttccaagaagcgcgggatgcccttgatggaaggcaattttttaagttcctcgtaggtgagctcttcaggggagctgagcccgtgctctgaaagggcccagtctgcaagatgagggttggaagcgacgaatgagctccacaggtcacgggccattagcatttgcaggtggtcgcgaaaggtcctaaactggcgacctatggccattttttctggggtgatgcagtagaaggtaagcgggtcttgttcccagcggtcccatccaaggttcgcggctaggtctcgcgcggcagtcactagaggctcatctccgccgaacttcatgaccagcatgaagggcacgagctgcttcccaaaggcccccatccaagtataggtctctacatcgtaggtgacaaagagacgctcggtgcgaggatgcgagccgatcgggaagaactggatctcccgccaccaattggaggagtggctattgatgtggtgaaagtagaagtccctgcgacgggccgaacactcgtgctggcttttgtaaaaacgtgcgcagtactggcagcggtgcacgggctgtacatcctgcacgaggttgacctgacgaccgcgcacaaggaagcagagtgggaatttgagcccctcgcctggcgggtttggctggtggtcttctacttcggctgcttgtccttgaccgtctggctgctcgaggggagttacggtggatcggaccaccacgccgcgcgagcccaaagtccagatgtccgcgcgcggcggtcggagcttgatgacaacatcgcgcagatgggagctgtccatggtctggagctcccgcggcgtcaggtcaggcgggagctcctgcaggtttacctcgcatagacgggtcagggcgcgggctagatccaggtgatacctaatttccaggggctggttggtggcggcgtcgatggcttgcaagaggccgcatccccgcggcgcgactacggtaccgcgcggcgggcggtgggccgcgggggtgtccttggatgatgcatctaaaagcggtgacgcgggcgagcccccggaggtagggggggctccggacccgccgggagagggggcaggggcacgtcggcgccgcgcgcgggcaggagctggtgctgcgcgcgtaggttgctggcgaacgcgacgacgcggcggttgatctcctgaatctggcgcctctgcgtgaagacgacgggcccggtgagcttgagcctgaaagagagttcgacagaatcaatttcggtgtcgttgacggcggcctggcgcaaaatctcctgcacgtctcctgagttgtcttgataggcgatctcggccatgaactgctcgatctcttcctcctggagatctccgcgtccggctcgctccacggtggcggcgaggtcgttggaaatgcgggccatgagctgcgagaaggcgttgaggcctccctcgttccagacgcggctgtagaccacgcccccttcggcatcgcgggcgcgcatgaccacctgcgcgagattgagctccacgtgccgggcgaagacggcgtagtttcgcaggcgctgaaagaggtagttgagggtggtggcggtgtgttctgccacgaagaagtacataacccagcgtcgcaacgtggattcgttgatatcccccaaggcctcaaggcgctccatggcctcgtagaagtccacggcgaagttgaaaaactgggagttgcgcgccgacacggttaactcctcctccagaagacggatgagctcggcgacagtgtcgcgcacctcgcgctcaaaggctacaggggcctcttcttcttcttcaatctcctcttccataagggcctccccttcttcttcttctggcggcggtgggggaggggggacacggcggcgacgacggcgcaccgggaggcggtcgacaaagcgctcgatcatctccccgcggcgacggcgcatggtctcggtgacggcgcggccgttctcgcgggggcgcagttggaagacgccgcccgtcatgtcccggttatgggttggcggggggctgccatgcggcagggatacggcgctaacgatgcatctcaacaattgttgtgtaggtactccgccgccgagggacctgagcgagtccgcatcgaccggatcggaaaacctctcgagaaaggcgtctaaccagtcacagtcgcaaggtaggctgagcaccgtggcgggcggcagcgggcggcggtcggggttgtttctggcggaggtgctgctgatgatgtaattaaagtaggcggtcttgagacggcggatggtcgacagaagcaccatgtccttgggtccggcctgctgaatgcgcaggcggtcggccatgccccaggcttcgttttgacatcggcgcaggtctttgtagtagtcttgcatgagcctttctaccggcacttcttcttctccttcctcttgtcctgcatctcttgcatctatcgctgcggcggcggcggagtttggccgtaggtggcgccctcttcctcccatgcgtgtgaccccgaagcccctcatcggctgaagcagggctaggtcggcgacaacgcgctcggctaatatggcctgctgcacctgcgtgagggtagactggaagtcatccatgtccacaaagcggtggtatgcgcccgtgttgatggtgtaagtgcagttggccataacggaccagttaacggtctggtgacccggctgcgagagctcggtgtacctgagacgcgagtaagccctcgagtcaaatacgtagtcgttgcaagtccgcaccaggtactggtatcccaccaaaaagtgcggcggcggctggcggtagaggggccagcgtagggtggccggggctccgggggcgagatcttccaacataaggcgatgatatccgtagatgtacctggacatccaggtgatgccggcggcggtggtggaggcgcgcggaaagtcgcggacgcggttccagatgttgcgcagcggcaaaaagtgctccatggtcgggacgctctggccggtcaggcgcgcgcaatcgttgacgctctaccgtgcaaaaggagagcctgtaagcgggcactcttccgtggtctggtggataaattcgcaagggtatcatggcggacgaccggggttcgagccccgtatccggccgtccgccgtgatccatgcggttaccgcccgcgtgtcgaacccaggtgtgcgacgtcagacaacgggggagtgctccttttggcttccttccaggcgcggcggctgctgcgctagcttttttggccactggccgcgcgcagcgtaagcggttaggctggaaagcgaaagcattaagtggctcgctccctgtagccggagggttattttccaagggttgagtcgcgggacccccggttcgagtctcggaccggccggactgcggcgaacgggggtttgcctccccgtcatgcaagaccccgcttgcaaattcctccggaaacagggacgagccccttttttgcttttcccagatgcatccggtgctgcggcagatgcgcccccctcctcagcagcggcaagagcaagagcagcggcagacatgcagggcaccctcccctcctcctaccgcgtcaggaggggcgacatccgcggttgacgcggcagcagatggtgattacgaacccccgcggcgccgggcccggcactacctggacttggaggagggcgagggcctggcgcggctaggagcgccctctcctgagcggtacccaagggtgcagctgaagcgtgatacgcgtgaggcgtacgtgccgcggcagaacctgtttcgcgaccgcgagggagaggagcccgaggagatgcgggatcgaaagttccacgcagggcgcgagctgcggcatggcctgaatcgcgagcggttgctgcgcgaggaggactttgagcccgacgcgcgaaccgggattagtcccgcgcgcgcacacgtggcggccgccgacctggtaaccgcatacgagcagacggtgaaccaggagattaactttcaaaaaagctttaacaaccacgtgcgtacgcttgtggcgcgcgaggaggtggctataggactgatgcatctgtgggactttgtaagcgcgctggagcaaaacccaaatagcaagccgctcatggcgcagctgttccttatagtgcagcacagcagggacaacgaggcattcagggatgcgctgctaaacatagtagagcccgagggccgctggctgctcgatttgataaacatcctgcagagcatagtggtgcaggagcgcagcttgagcctggctgacaaggtggccgccatcaactattccatgcttagcctgggcaagttttacgcccgcaagatataccataccccttacgttcccatagacaaggaggtaaagatcgaggggttctacatgcgcatggcgctgaaggtgcttaccttgagcgacgacctgggcgtttatcgcaacgagcgcatccacaaggccgtgagcgtgagccggcggcgcgagctcagcgaccgcgagctgatgcacagcctgcaaagggccctggctggcacgggcagcggcgatagagaggccgagtcctactttgacgcgggcgctgacctgcgctgggccccaagccgacgcgccctggaggcagctggggccggacctgggctggcggtggcacccgcgcgcgctggcaacgtcggcggcgtggaggaatatgacgaggacgatgagtacgagccagaggacggcgagtactaagcggtgatgtttctgatcagatgatgcaagacgcaacggacccggcggtgcgggcggcgctgcagagccagccgtccggccttaactccacggacgactggcgccaggtcatggaccgcatcatgtcgctgactgcgcgcaatcctgacgcgttccggcagcagccgcaggccaaccggctctccgcaattctggaagcggtggtcccggcgcgcgcaaaccccacgcacgagaaggtgctggcgatcgtaaacgcgctggccgaaaacagggccatccggcccgacgaggccggcctggtctacgacgcgctgcttcagcgcgtggctcgttacaacagcggcaacgtgcagaccaacctggaccggctggtgggggatgtgcgcgaggccgtggcgcagcgtgagcgcgcgcagcagcagggcaacctgggctccatggttgcactaaacgccttcctgagtacacagcccgccaacgtgccgcggggacaggaggactacaccaactttgtgagcgcactgcggctaatggtgactgagacaccgcaaagtgaggtgtaccagtctgggccagactattttttccagaccagtagacaaggcctgcagaccgtaaacctgagccaggctttcaaaaacttgcaggggctgtggggggtgcgggctcccacaggcgaccgcgcgaccgtgtctagcttgctgacgcccaactcgcgcctgttgctgctgctaatagcgcccttcacggacagtggcagcgtgtcccgggacacatacctaggtcacttgctgacactgtaccgcgaggccataggtcaggcgcatgtggacgagcatactttccaggagattacaagtgtcagccgcgcgctggggcaggaggacacgggcagcctggaggcaaccctaaactacctgctgaccaaccggcggcagaagatcccctcgttgcacagtttaaacagcgaggaggagcgcattttgcgctacgtgcagcagagcgtgagccttaacctgatgcgcgacggggtaacgcccagcgtggcgctggacatgaccgcgcgcaacatggaaccgggcatgtatgcctcaaaccggccgtttatcaaccgcctaatggactacttgcatcgcgcggccgccgtgaaccccgagtatttcaccaatgccatcttgaacccgcactggctaccgccccctggtttctacaccgggggattcgaggtgcccgagggtaacgatggattcctctgggacgacatagacgacagcgtgttttccccgcaaccgcagaccctgctagagttgcaacagcgcgagcaggcagaggcggcgctgcgaaaggaaagcttccgcaggccaagcagcttgtccgatctaggcgctgcggccccgcggtcagatgctagtagcccatttccaagcttgatagggtctcttaccagcactcgcaccacccgcccgcgcctgctgggcgaggaggagtacctaaacaactcgctgctgcagccgcagcgcgaaaaaaacctgcctccggcatttcccaacaacgggatagagagcctagtggacaagatgagtagatggaagacgtacgcgcaggagcacagggacgtgccaggcccgcgcccgcccacccgtcgtcaaaggcacgaccgtcagcggggtctggtgtgggaggacgatgactcggcagacgacagcagcgtcctggatttgggagggagtggcaacccgtttgcgcaccttcgccccaggctggggagaatgttttaaaaaaaaaaaagcatgatgcaaaataaaaaactcaccaaggccatggcaccgagcgttggttttcttgtattccccttagtatgcggcgcgcggcgatgtatgaggaaggtcctcctccctcctacgagagtgtggtgagcgcggcgccagtggcggcggcgctgggttctcccttcgatgctcccctggacccgccgtttgtgcctccgcggtacctgcggcctaccggggggagaaacagcatccgttactctgagttggcacccctattcgacaccacccgtgtgtacctggtggacaacaagtcaacggatgtggcatccctgaactaccagaacgaccacagcaactttctgaccacggtcattcaaaacaatgactacagcccgggggaggcaagcacacagaccatcaatcttgacgaccggtcgcactggggcggcgacctgaaaaccatcctgcataccaacatgccaaatgtgaacgagttcatgtttaccaataagtttaaggcgcgggtgatggtgtcgcgcttgcctactaaggacaatcaggtggagctgaaatacgagtgggtggagttcacgctgcccgagggcaactactccgagaccatgaccatagaccttatgaacaacgcgatcgtggagcactacttgaaagtgggcagacagaacggggttctggaaagcgacatcggggtaaagtttgacacccgcaacttcagactggggtttgaccccgtcactggtcttgtcatgcctggggtatatacaaacgaagccttccatccagacatcattttgctgccaggatgcggggtggacttcacccacagccgcctgagcaacttgttgggcatccgcaagcggcaacccttccaggagggctttaggatcacctacgatgatctggagggtggtaacattcccgcactgttggatgtggacgcctaccaggcgagcttgaaagatgacaccgaacagggcgggggtggcgcaggcggcagcaacagcagtggcagcggcgcggaagagaactccaacgcggcagccgcggcaatgcagccggtggaggacatgaacgatcatgccattcgcggcgacacctttgccacacgggctgaggagaagcgcgctgaggccgaagcagcggccgaagctgccgcccccgctgcgcaacccgaggtcgagaagcctcagaagaaaccggtgatcaaacccctgacagaggacagcaagaaacgcagttacaacctaataagcaatgacagcaccttcacccagtaccgcagctggtaccttgcatacaactacggcgaccctcagaccggaatccgctcatggaccctgctttgcactcctgacgtaacctgcggctcggagcaggtctactggtcgttgccagacatgatgcaagaccccgtgaccttccgctccacgcgccagatcagcaactttccggtggtgggcgccgagctgttgcccgtgcactccaagagcttctacaacgaccaggccgtctactcccaactcatccgccagtttacctctctgacccacgtgttcaatcgctttcccgagaaccagattttggcgcgcccgccagcccccaccatcaccaccgtcagtgaaaacgttcctgctctcacagatcacgggacgctaccgctgcgcaacagcatcggaggagtccagcgagtgaccattactgacgccagacgccgcacctgcccctacgtttacaaggccctgggcatagtctcgccgcgcgtcctatcgagccgcactttttgagcaagcatgtccatccttatatcgcccagcaataacacaggctggggcctgcgcttcccaagcaagatgtttggcggggccaagaagcgctccgaccaacacccagtgcgcgtgcgcgggcactaccgcgcgccctggggcgcgcacaaacgcggccgcactgggcgcaccaccgtcgatgacgccatcgacgcggtggtggaggaggcgcgcaactacacgcccacgccgccaccagtgtccacagtggacgcggccattcagaccgtggtgcgcggagcccggcgctatgctaaaatgaagagacggcggaggcgcgtagcacgtcgccaccgccgccgacccggcactgccgcccaacgcgcggcggcggccctgcttaaccgcgcacgtcgcaccggccgacgggcggccatgcgggccgctcgaaggctggccgcgggtattgtcactgtgccccccaggtccaggcgacgagcggccgccgcagcagccgcggccattagtgctatgactcagggtcgcaggggcaacgtgtattgggtgcgcgactcggttagcggcctgcgcgtgcccgtgcgcacccgccccccgcgcaactagattgcaagaaaaaactacttagactcgtactgttgtatgtatccagcggcggcggcgcgcaacgaagctatgtccaagcgcaaaatcaaagaagagatgctccaggtcatcgcgccggagatctatggccccccgaagaaggaagagcaggattacaagccccgaaagctaaagcgggtcaaaaagaaaaagaaagatgatgatgatgaacttgacgacgaggtggaactgctgcacgctaccgcgcccaggcgacgggtacagtggaaaggtcgacgcgtaaaacgtgttttgcgacccggcaccaccgtagtctttacgcccggtgagcgctccacccgcacctacaagcgcgtgtatgatgaggtgtacggcgacgaggacctgcttgagcaggccaacgagcgcctcggggagtttgcctacggaaagcggcataaggacatgctggcgttgccgctggacgagggcaacccaacacctagcctaaagcccgtaacactgcagcaggtgctgcccgcgcttgcaccgtccgaagaaaagcgcggcctaaagcgcgagtctggtgacttggcacccaccgtgcagctgatggtacccaagcgccagcgactggaagatgtcttggaaaaaatgaccgtggaacctgggctggagcccgaggtccgcgtgcggccaatcaagcaggtggcgccgggactgggcgtgcagaccgtggacgttcagatacccactaccagtagcaccagtattgccaccgccacagagggcatggagacacaaacgtccccggttgcctcagcggtggcggatgccgcggtgcaggcggtcgctgcggccgcgtccaagacctctacggaggtgcaaacggacccgtggatgtttcgcgtttcagccccccggcgcccgcgcggttcgaggaagtacggcgccgccagcgcgctactgcccgaatatgccctacatccttccattgcgcctacccccggctatcgtggctacacctaccgccccagaagacgagcaactacccgacgccgaaccaccactggaacccgccgccgccgtcgccgtcgccagcccgtgctggccccgatttccgtgcgcagggtggctcgcgaaggaggcaggaccctggtgctgccaacagcgcgctaccaccccagcatcgtttaaaagccggtctttgtggttcttgcagatatggccctcacctgccgcctccgtttcccggtgccgggattccgaggaagaatgcaccgtaggaggggcatggccggccacggcctgacgggcggcatgcgtcgtgcgcaccaccggcggcggcgcgcgtcgcaccgtcgcatgcgcggcggtatcctgcccctccttattccactgatcgccgcggcgattggcgccgtgcccggaattgcatccgtggccttgcaggcgcagagacactgattaaaaacaagttgcatgtggaaaaatcaaaataaaaagtctggactctcacgctcgcttggtcctgtaactattttgtagaatggaagacatcaactttgcgtctctggccccgcgacacggctcgcgcccgttcatgggaaactggcaagatatcggcaccagcaatatgagcggtggcgccttcagctggggctcgctgtggagcggcattaaaaatttcggttccaccgttaagaactatggcagcaaggcctggaacagcagcacaggccagatgctgagggataagttgaaagagcaaaatttccaacaaaaggtggtagatggcctggcctctggcattagcggggtggtggacctggccaaccaggcagtgcaaaataagattaacagtaagcttgatccccgccctcccgtagaggagcctccaccggccgtggagacagtgtctccagaggggcgtggcgaaaagcgtccgcgccccgacagggaagaaactctggtgacgcaaatagacgagcctccctcgtacgaggaggcactaaagcaaggcctgcccaccacccgtcccatcgcgcccatggctaccggagtgctgggccagcacacacccgtaacgctggacctgcctccccccgccgacacccagcagaaacctgtgctgccaggcccgaccgccgttgttgtaacccgtcctagccgcgcgtccctgcgccgcgccgccagcggtccgcgatcgttgcggcccgtagccagtggcaactggcaaagcacactgaacagcatcgtgggtctgggggtgcaatccctgaagcgccgacgatgcttctgaatagctaacgtgtcgtatgtgtgtcatgtatgcgtccatgtcgccgccagaggagctgctgagccgccgcgcgcccgctttccaagatggctaccccttcgatgatgccgcagtggtcttacatgcacatctcgggccaggacgcctcggagtacctgagccccgggctggtgcagtttgcccgcgccaccgagacgtacttcagcctgaataacaagtttagaaaccccacggtggcgcctacgcacgacgtgaccacagaccggtcccagcgtttgacgctgcggttcatccctgtggaccgtgaggatactgcgtactcgtacaaggcgcggttcaccctagctgtgggtgataaccgtgtgctggacatggcttccacgtactttgacatccgcggcgtgctggacaggggccctacttttaagccctactctggcactgcctacaacgccctggctcccaagggtgccccaaatccttgcgaatgggatgaagctgctactgctcttgaaataaacctagaagaagaggacgatgacaacgaagacgaagtagacgagcaagctgagcagcaaaaaactcacgtatttgggcaggcgccttattctggtataaatattacaaaggagggtattcaaataggtgtcgaaggtcaaacacctaaatatgccgataaaacatttcaacctgaacctcaaataggagaatctcagtggtacgaaactgaaattaatcatgcagctgggagagtccttaaaaagactaccccaatgaaaccatgttacggttcatatgcaaaacccacaaatgaaaatggagggcaaggcattcttgtaaagcaacaaaatggaaagctagaaagtcaagtggaaatgcaatttttctcaactactgaggcgaccgcaggcaatggtgataacttgactcctaaagtggtattgtacagtgaagatgtagatatagaaaccccagacactcatatttcttacatgcccactattaaggaaggtaactcacgagaactaatgggccaacaatctatgcccaacaggcctaattacattgcttttagggacaattttattggtctaatgtattacaacagcacgggtaatatgggtgttctggcgggccaagcatcgcagttgaatgctgttgtagatttgcaagacagaaacacagagctttcataccagcttttgcttgattccattggtgatagaaccaggtacttttctatgtggaatcaggctgttgacagctatgatccagatgttagaattattgaaaatcatggaactgaagatgaacttccaaattactgctttccactgggaggtgtgattaatacagagactcttaccaaggtaaaacctaaaacaggtcaggaaaatggatgggaaaaagatgctacagaattttcagataaaaatgaaataagagttggaaataattttgccatggaaatcaatctaaatgccaacctgtggagaaatttcctgtactccaacatagcgctgtatttgcccgacaagctaaagtacagtccttccaacgtaaaaatttctgataacccaaacacctacgactacatgaacaagcgagtggtggctcccgggttagtggactgctacattaaccttggagcacgctggtcccttgactatatggacaacgtcaacccatttaaccaccaccgcaatgctggcctgcgctaccgctcaatgttgctgggcaatggtcgctatgtgcccttccacatccaggtgcctcagaagttctttgccattaaaaacctccttctcctgccgggctcatacacctacgagtggaacttcaggaaggatgttaacatggttctgcagagctccctaggaaatgacctaagggttgacggagccagcattaagtttgatagcatttgcctttacgccaccttcttccccatggcccacaacaccgcctccacgcttgaggccatgcttagaaacgacaccaacgaccagtcctttaacgactatctctccgccgccaacatgctctaccctatacccgccaacgctaccaacgtgcccatatccatcccctcccgcaactgggcggctttccgcggctgggccttcacgcgccttaagactaaggaaaccccatcactgggctcgggctacgacccttattacacctactctggctctataccctacctagatggaaccttttacctcaaccacacctttaagaaggtggccattacctttgactcttctgtcagctggcctggcaatgaccgcctgcttacccccaacgagtttgaaattaagcgctcagttgacggggagggttacaacgttgcccagtgtaacatgaccaaagactggttcctggtacaaatgctagctaactacaacattggctaccagggcttctatatcccagagagctacaaggaccgcatgtactccttctttagaaacttccagcccatgagccgtcaggtggtggatgatactaaatacaaggactaccaacaggtgggcatcctacaccaacacaacaactctggatttgttggctaccttgcccccaccatgcgcgaaggacaggcctaccctgctaacttcccctatccgcttataggcaagaccgcagttgacagcattacccagaaaaagtttctttgcgatcgcaccctttggcgcatcccattctccagtaactttatgtccatgggcgcactcacagacctgggccaaaaccttctctacgccaactccgcccacgcgctagacatgacttttgaggtggatcccatggacgagcccacccttctttatgttttgtttgaagtctttgacgtggtccgtgtgcaccggccgcaccgcggcgtcatcgaaaccgtgtacctgcgcacgcccttctcggccggcaacgccacaacataaagaagcaagcaacatcaacaacagctgccgccatgggctccagtgagcaggaactgaaagccattgtcaaagatcttggttgtgggccatattttttgggcacctatgacaagcgctttccaggctttgtttctccacacaagctcgcctgcgccatagtcaatacggccggtcgcgagactgggggcgtacactggatggcctttgcctggaacccgcactcaaaaacatgctacctctttgagccctttggcttttctgaccagcgactcaagcaggtttaccagtttgagtacgagtcactcctgcgccgtagcgccattgcttcttcccccgaccgctgtataacgctggaaaagtccacccaaagcgtacaggggcccaactcggccgcctgtggactattctgctgcatgtttctccacgcctttgccaactggccccaaactcccatggatcacaaccccaccatgaaccttattaccggggtacccaactccatgctcaacagtccccaggtacagcccaccctgcgtcgcaaccaggaacagctctacagcttcctggagcgccactcgccctacttccgcagccacagtgcgcagattaggagcgccacttctttttgtcacttgaaaaacatgtaaaaataatgtactagagacactttcaataaaggcaaatgcttttatttgtacactctcgggtgattatttacccccacccttgccgtctgcgccgtttaaaaatcaaaggggttctgccgcgcatcgctatgcgccactggcagggacacgttgcgatactggtgtttagtgctccacttaaactcaggcacaaccatccgcggcagctcggtgaagttttcactccacaggctgcgcaccatcaccaacgcgtttagcaggtcgggcgccgatatcttgaagtcgcagttggggcctccgccctgcgcgcgcgagttgcgatacacagggttgcagcactggaacactatcagcgccgggtggtgcacgctggccagcacgctcttgtcggagatcagatccgcgtccaggtcctccgcgttgctcagggcgaacggagtcaactttggtagctgccttcccaaaaagggcgcgtgcccaggctttgagttgcactcgcaccgtagtggcatcaaaaggtgaccgtgcccggtctgggcgttaggatacagcgcctgcataaaagccttgatctgcttaaaagccacctgagcctttgcgccttcagagaagaacatgccgcaagacttgccggaaaactgattggccggacaggccgcgtcgtgcacgcagcaccttgcgtcggtgttggagatctgcaccacatttcggccccaccggttcttcacgatcttggccttgctagactgctccttcagcgcgcgctgcccgttttcgctcgtcacatccatttcaatcacgtgctccttatttatcataatgcttccgtgtagacacttaagctcgccttcgatctcagcgcagcggtgcagccacaacgcgcagcccgtgggctcgtgatgcttgtaggtcacctctgcaaacgactgcaggtacgcctgcaggaatcgccccatcatcgtcacaaaggtcttgttgctggtgaaggtcagctgcaacccgcggtgctcctcgttcagccaggtcttgcatacggccgccagagcttccacttggtcaggcagtagtttgaagttcgcctttagatcgttatccacgtggtacttgtccatcagcgcgcgcgcagcctccatgcccttctcccacgcagacacgatcggcacactcagcgggttcatcaccgtaatttcactttccgcttcgctgggctcttcctcttcctcttgcgtccgcataccacgcgccactgggtcgtcttcattcagccgccgcactgtgcgcttacctcctttgccatgcttgattagcaccggtgggttgctgaaacccaccatttgtagcgccacatcttctctttcttcctcgctgtccacgattacctctggtgatggcgggcgctcgggcttgggagaagggcgcttctttttcttcttgggcgcaatggccaaatccgccgccgaggtcgatggccgcgggctgggtgtgcgcggcaccagcgcgtcttgtgatgagtcttcctcgtcctcggactcgatacgccgcctcatccgcttttttgggggcgcccggggaggcggcggcgacggggacggggacgacacgtcctccatggttgggggacgtcgcgccgcaccgcgtccgcgctcgggggtggtttcgcgctgctcctcttcccgactggccatttccttctcctataggcagaaaaagatcatggagtcagtcgagaagaaggacagcctaaccgccccctctgagttcgccaccaccgcctccaccgatgccgccaacgcgcctaccaccttccccgtcgaggcacccccgcttgaggaggaggaagtgattatcgagcaggacccaggttttgtaagcgaagacgacgaggaccgctcagtaccaacagaggataaaaagcaagaccaggacaacgcagaggcaaacgaggaacaagtcgggcggggggacgaaaggcatggcgactacctagatgtgggagacgacgtgctgttgaagcatctgcagcgccagtgcgccattatctgcgacgcgttgcaagagcgcagcgatgtgcccctcgccatagcggatgtcagccttgcctacgaacgccacctattctcaccgcgcgtaccccccaaacgccaagaaaacggcacatgcgagcccaacccgcgcctcaacttctaccccgtatttgccgtgccagaggtgcttgccacctatcacatctttttccaaaactgcaagatacccctatcctgccgtgccaaccgcagccgagcggacaagcagctggccttgcggcagggcgctgtcatacctgatatcgcctcgctcaacgaagtgccaaaaatctttgagggtcttggacgcgacgagaagcgcgcggcaaacgctctgcaacaggaaaacagcgaaaatgaaagtcactctggagtgttggtggaactcgagggtgacaacgcgcgcctagccgtactaaaacgcagcatcgaggtcacccactttgcctacccggcacttaacctaccccccaaggtcatgagcacagtcatgagtgagctgatcgtgcgccgtgcgcagcccctggagagggatgcaaatttgcaagaacaaacagaggagggcctacccgcagttggcgacgagcagctagcgcgctggcttcaaacgcgcgagcctgccgacttggaggagcgacgcaaactaatgatggccgcagtgctcgttaccgtggagcttgagtgcatgcagcggttctttgctgacccggagatgcagcgcaagctagaggaaacattgcactacacctttcgacagggctacgtacgccaggcctgcaagatctccaacgtggagctctgcaacctggtctcctaccttggaattttgcacgaaaaccgccttgggcaaaacgtgcttcattccacgctcaagggcgaggcgcgccgcgactacgtccgcgactgcgtttacttatttctatgctacacctggcagacggccatgggcgtttggcagcagtgcttggaggagtgcaacctcaaggagctgcagaaactgctaaagcaaaacttgaaggacctatggacggccttcaacgagcgctccgtggccgcgcacctggcggacatcattttccccgaacgcctgcttaaaaccctgcaacagggtctgccagacttcaccagtcaaagcatgttgcagaactttaggaactttatcctagagcgctcaggaatcttgcccgccacctgctgtgcacttcctagcgactttgtgcccattaagtaccgcgaatgccctccgccgctttggggccactgctaccttctgcagctagccaactaccttgcctaccactctgacataatggaagacgtgagcggtgacggtctactggagtgtcactgtcgctgcaacctatgcaccccgcaccgctccctggtttgcaattcgcagctgcttaacgaaagtcaaattatcggtacctttgagctgcagggtccctcgcctgacgaaaagtccgcggctccggggttgaaactcactccggggctgtggacgtcggcttaccttcgcaaatttgtacctgaggactaccacgcccacgagattaggttctacgaagaccaatcccgcccgccaaatgcggagcttaccgcctgcgtcattacccagggccacattcttggccaattgcaagccatcaacaaagcccgccaagagtttctgctacgaaagggacggggggtttacttggacccccagtccggcgaggagctcaacccaatccccccgccgccgcagccctatcagcagcagccgcgggcccttgcttcccaggatggcacccaaaaagaagctgcagctgccgccgccacccacggacgaggaggaatactgggacagtcaggcagaggaggttttggacgaggaggaggaggacatgatggaagactgggagagcctagacgaggaagcttccgaggtcgaagaggtgtcagacgaaacaccgtcaccctcggtcgcattcccctcgccggcgccccagaaatcggcaaccggttccagcatggctacaacctccgctcctcaggcgccgccggcactgcccgttcgccgacccaaccgtagatgggacaccactggaaccagggccggtaagtccaagcagccgccgccgttagcccaagagcaacaacagcgccaaggctaccgctcatggcgcgggcacaagaacgccatagttgcttgcttgcaagactgtgggggcaacatctccttcgcccgccgctttcttctctaccatcacggcgtggccttcccccgtaacatcctgcattactaccgtcatctctacagcccatactgcaccggcggcagcggcagcggcagcaacagcagcggccacacagaagcaaaggcgaccggatagcaagactctgacaaagcccaagaaatccacagcggcggcagcagcaggaggaggagcgctgcgtctggcgcccaacgaacccgtatcgacccgcgagcttagaaacaggatttttcccactctgtatgctatatttcaacagagcaggggccaagaacaagagctgaaaataaaaaacaggtctctgcgatccctcacccgcagctgcctgtatcacaaaagcgaagatcagcttcggcgcacgctggaagacgcggaggctctcttcagtaaatactgcgcgctgactcttaaggactagtttcgcgccctttctcaaatttaagcgcgaaaactacgtcatctccagcggccacacccggcgccagcacctgtcgtcagcgccattatgagcaaggaaattcccacgccctacatgtggagttaccagccacaaatgggacttgcggctggagctgcccaagactactcaacccgaataaactacatgagcgcgggaccccacatgatatcccgggtcaacggaatccgcgcccaccgaaaccgaattctcttggaacaggcggctattaccaccacacctcgtaataaccttaatccccgtagttggcccgctgccctggtgtaccaggaaagtcccgctcccaccactgtggtacttcccagagacgcccaggccgaagttcagatgactaactcaggggcgcagcttgcgggcggctttcgtcacagggtgcggtcgcccgggcagggtataactcacctgacaatcagagggcgaggtattcagctcaacgacgagtcggtgagctcctcgcttggtctccgtccggacgggacatttcagatcggcggcgccggccgtccttcattcacgcctcgtcaggcaatcctaactctgcagacctcgtcctctgagccgcgctctggaggcattggaactctgcaatttattgaggagtttgtgccatcggtctactttaaccccttctcgggacctcccggccactatccggatcaatttattcctaactttgacgcggtaaaggactcggcggacggctacgactgaatgttaagtggagaggcagagcaactgcgcctgaaacacctggtccactgtcgccgccacaagtgctttgcccgcgactccggtgagttttgctactttgaattgcccgaggatcatatcgagggcccggcgcacggcgtccggcttaccgcccagggagagcttgcccgtagcctgattcgggagtttacccagcgccccctgctagttgagcgggacaggggaccctgtgttctcactgtgatttgcaactgtcctaaccttggattacatcaagatcctctagttataactagagtacccggggatcttattccctttaactaataaaaaaaaataataaagcatcacttacttaaaatcagttagcaaatttctgtccagtttattcagcagcacctccttgccctcctcccagctctggtattgcagcttcctcctggctgcaaactttctccacaatctaaatggaatgtcagtttcctcctgttcctgtccatccgcacccactatcttcatgttgttgcagatgaagcgcgcaagaccgtctgaagataccttcaaccccgtgtatccatatgacacggaaaccggtcctccaactgtgccttttcttactcctccctttgtatcccccaatgggtttcaagagagtccccctggggtactctctttgcgcctatccgaacctctagttacctccaatggcatgcttgcgctcaaaatgggcaacggcctctctctggacgaggccggcaaccttacctcccaaaatgtaaccactgtgagcccacctctcaaaaaaaccaagtcaaacataaacctggaaatatctgcacccctcacagttacctcagaagccctaactgtggctgccgccgcacctctaatggtcgcgggcaacacactcaccatgcaatcacaggccccgctaaccgtgcacgactccaaacttagcattgccacccaaggacccctcacagtgtcagaaggaaagctagccctgcaaacatcaggccccctcaccaccaccgatagcagtacccttactatcactgcctcaccccctctaactactgccactggtagcttgggcattgacttgaaagagcccatttatacacaaaatggaaaactaggactaaagtacggggctcctttgcatgtaacagacgacctaaacactttgaccgtagcaactggtccaggtgtgactattaataatacttccttgcaaactaaagttactggagccttgggttttgattcacaaggcaatatgcaacttaatgtagcaggaggactaaggattgattctcaaaacagacgccttatacttgatgttagttatccgtttgatgctcaaaaccaactaaatctaagactaggacagggccctctttttataaactcagcccacaacttggatattaactacaacaaaggcctttacttgtttacagcttcaaacaattccaaaaagcttgaggttaacctaagcactgccaaggggttgatgtttgacgctacagccatagccattaatgcaggagatgggcttgaatttggttcacctaatgcaccaaacacaaatcccctcaaaacaaaaattggccatggcctagaatttgattcaaacaaggctatggttcctaaactaggaactggccttagttttgacagcacaggtgccattacagtaggaaacaaaaataatgataagctaactttgtggaccacaccagctccatctcctaactgtagactaaatgcagagaaagatgctaaactcactttggtcttaacaaaatgtggcagtcaaatacttgctacagtttcagttttggctgttaaaggcagtttggctccaatatctggaacagttcaaagtgctcatcttattataagatttgacgaaaatggagtgctactaaacaattccttcctggacccagaatattggaactttagaaatggagatcttactgaaggcacagcctatacaaacgctgttggatttatgcctaacctatcagcttatccaaaatctcacggtaaaactgccaaaagtaacattgtcagtcaagtttacttaaacggagacaaaactaaacctgtaacactaaccattacactaaacggtacacaggaaacaggagacacaactccaagtgcatactctatgtcattttcatgggactggtctggccacaactacattaatgaaatatttgccacatcctcttacactttttcatacattgcccaagaataaagaatcgtttgtgttatgtttcaacgtgtttatttttcaattgcagaaaatttcaagtcatttttcattcagtagtatagccccaccaccacatagcttatacagatcaccgtaccttaatcaaactcacagaaccctagtattcaacctgccacctccctcccaacacacagagtacacagtcctttctccccggctggccttaaaaagcatcatatcatgggtaacagacatattcttaggtgttatattccacacggtttcctgtcgagccaaacgctcatcagtgatattaataaactccccgggcagctcacttaagttcatgtcgctgtccagctgctgagccacaggctgctgtccaacttgcggttgcttaacgggcggcgaaggagaagtccacgcctacatgggggtagagtcataatcgtgcatcaggatagggcggtggtgctgcagcagcgcgcgaataaactgctgccgccgccgctccgtcctgcaggaatacaacatggcagtggtctcctcagcgatgattcgcaccgcccgcagcataaggcgccttgtcctccgggcacagcagcgcaccctgatctcacttaaatcagcacagtaactgcagcacagcaccacaatattgttcaaaatcccacagtgcaaggcgctgtatccaaagctcatggcggggaccacagaacccacgtggccatcataccacaagcgcaggtagattaagtggcgacccctcataaacacgctggacataaacattacctcttttggcatgttgtaattcaccacctcccggtaccatataaacctctgattaaacatggcgccatccaccaccatcctaaaccagctggccaaaacctgcccgccggctatacactgcagggaaccgggactggaacaatgacagtggagagcccaggactcgtaaccatggatcatcatgctcgtcatgatatcaatgttggcacaacacaggcacacgtgcatacacttcctcaggattacaagctcctcccgcgttagaaccatatcccagggaacaacccattcctgaatcagcgtaaatcccacactgcagggaagacctcgcacgtaactcacgttgtgcattgtcaaagtgttacattcgggcagcagcggatgatcctccagtatggtagcgcgggtttctgtctcaaaaggaggtagacgatccctactgtacggagtgcgccgagacaaccgagatcgtgttggtcgtagtgtcatgccaaatggaacgccggacgtagtcatatttcctgaagcaaaaccaggtgcgggcgtgacaaacagatctgcgtctccggtctcgccgcttagatcgctctgtgtagtagttgtagtatatccactctctcaaagcatccaggcgccccctggcttcgggttctatgtaaactccttcatgcgccgctgccctgataacatccaccaccgcagaataagccacacccagccaacctacacattcgttctgcgagtcacacacgggaggagcgggaagagctggaagaaccatgtttttttttttattccaaaagattatccaaaacctcaaaatgaagatctattaagtgaacgcgctcccctccggtggcgtggtcaaactctacagccaaagaacagataatggcatttgtaagatgttgcacaatggcttccaaaaggcaaacggccctcacgtccaagtggacgtaaaggctaaacccttcagggtgaatctcctctataaacattccagcaccttcaaccatgcccaaataattctcatctcgccaccttctcaatatatctctaagcaaatcccgaatattaagtccggccattgtaaaaatctgctccagagcgccctccaccttcagcctcaagcagcgaatcatgattgcaaaaattcaggttcctcacagacctgtataagattcaaaagcggaacattaacaaaaataccgcgatcccgtaggtcccttcgcagggccagctgaacataatcgtgcaggtctgcacggaccagcgcggccacttccccgccaggaaccttgacaaaagaacccacactgattatgacacgcatactcggagctatgctaaccagcgtagccccgatgtaagctttgttgcatgggcggcgatataaaatgcaaggtgctgctcaaaaaatcaggcaaagcctcgcgcaaaaaagaaagcacatcgtagtcatgctcatgcagataaaggcaggtaagctccggaaccaccacagaaaaagacaccatttttctctcaaacatgtctgcgggtttctgcataaacacaaaataaaataacaaaaaaacatttaaacattagaagcctgtcttacaacaggaaaaacaacccttataagcataagacggactacggccatgccggcgtgaccgtaaaaaaactggtcaccgtgattaaaaagcaccaccgacagctcctcggtcatgtccggagtcataatgtaagactcggtaaacacatcaggttgattcatcggtcagtgctaaaaagcgaccgaaatagcccgggggaatacatacccgcaggcgtagagacaacattacagcccccataggaggtataacaaaattaataggagagaaaaacacataaacacctgaaaaaccctcctgcctaggcaaaatagcaccctcccgctccagaacaacatacagcgcttcacagcggcagcctaacagtcagccttaccagtaaaaaagaaaacctattaaaaaaacaccactcgacacggcaccagctcaatcagtcacagtgtaaaaaagggccaagtgcagagcgagtatatataggactaaaaaatgacgtaacggttaaagtccacaaaaaacacccagaaaaccgcacgcgaacctacgcccagaaacgaaagccaaaaaacccacaacttcctcaaatcgtcacttccgttttcccacgttacgtaacttcccattttaagaaaactacaattcccaacacatacaagttactccgccctaaaacctacgtcacccgccccgttcccacgccccgcgccacgtcacaaactccaccccctcattatcatattggcttcaatccaaaataaggtatattattgatgatnnnnnttaat

SEQ ID NO: 8 - DNA, 22 bp, Artificial Sequence
  synthetic nucleotide - forward primer for ND 1.1
gctcgctattgtgtctctagtg

SEQ ID NO: 9 - DNA, 21 bp, Artificial Sequence
  synthetic nucleotide - reverse primer for ND 1.1
tgtcttgggcatgagtaactg

SEQ ID NO: 10 - DNA, 26 bp, Artificial Sequence
  synhetic nucleotide - probe for ND 1.1
  misc_feature (1)..(1): 5' labeled with 56-FAM (carboxyfluorescein)
  misc_feature (9)..(10): ZEN (non-abbreviation) quencher incorporate between C (position 9) and T (position 10)
  misc_feature (26)..(26): 3' end labeled with 3IABkFQ (Iowa black fluorescein quencher)
tcgacctgctctgttgagttattggc

SEQ ID NO: 11 - DNA, 21 bp, Artificial Sequence
  short hairpin RNA adjuvant
gaaacgatatgggctgaatac